European Patent Specification EP 3 873 525 B1, published December 25, 2024. Title: COMPOSITIONS AND METHODS FOR TREATING BRAIN INJURY. Applicant: ANNEXON, INC. THE REGENTS OF THE UNIVERSITY OF CALIFORNIA. The sequence listing filed with the application follows.

SEQUENCE LISTING (72 sequences)

SEQ ID NO: 1 - protein, 245 aa, Homo sapiens
MEGPRGWLVLCVLAISLASMVTEDLCRAPDGKKGEAGRPGRRGRPGLKGEQGEPGAPGIRTGIQGLKGDQGEPGPSGNPGKVGYPGPSGPLGARGIPGIKGTKGSPGNIKDQPRPAFSAIRRNPPMGGNVVIFDTVITNQEEPYQNHSGRFVCTVPGYYYFTFQVLSQWEICLSIVSSSRGQVRRSLGFCDTTNKGLFQVVSGGMVLQLQQGDQVWVEKDPKKGHIYQGSEADSVFSGFLIFPSA

SEQ ID NO: 2 - protein, 253 aa, Homo sapiens
MMMKIPWGSIPVLMLLLLLGLIDISQAQLSCTGPPAIPGIPGIPGTPGPDGQPGTPGIKGEKGLPGLAGDHGEFGEKGDPGIPGNPGKVGPKGPMGPKGGPGAPGAPGPKGESGDYKATQKIAFSATRTINVPLRRDQTIRFDHVITNMNNNYEPRSGKFTCKVPGLYYFTYHASSRGNLCVNLMRGRERAQKVVTFCDYAYNTFQVTTGGMVLKLEQGENVFLQATDKNSLLGMEGANSIFSGFLLFPDMEA

SEQ ID NO: 3 - protein, 245 aa, Homo sapiens
MDVGPSSLPHLGLKLLLLLLLLPLRGQANTGCYGIPGMPGLPGAPGKDGYDGLPGPKGEPGIPAIPGIRGPKGQKGEPGLPGHPGKNGPMGPPGMPGVPGPMGIPGEPGEEGRYKQKFQSVFTVTRQTHQPPAPNSLIRFNAVLTNPQGDYDTSTGKFTCKVPGLYYFVYHASHTANLCVLLYRSGVKVVTFCGHTSKTNQVNSGGVLLRLQVGEEVWLAVNDYYDMVGIQGSDSVFSGFLLFPD

SEQ ID NO: 4 - protein, 107 aa, Artificial Sequence
  Description of Artificial Sequence: Synthetic polypeptide
DVQITQSPSYLAASPGETITINCRASKSINKYLAWYQEKPGKTNKLLIYSGSTLQSGIPSRFSGSGSGTDFTLTISSLEPEDFAMYYCQQHNEYPLTFGAGTKLELK

SEQ ID NO: 5 - protein, 11 aa, Artificial Sequence
  Description of Artificial Sequence: Synthetic peptide
RASKSINKYLA

SEQ ID NO: 6 - protein, 7 aa, Artificial Sequence
  Description of Artificial Sequence: Synthetic peptide
SGSTLQS

SEQ ID NO: 7 - protein, 9 aa, Artificial Sequence
  Description of Artificial Sequence: Synthetic peptide
QQHNEYPLT

SEQ ID NO: 8 - protein, 121 aa, Artificial Sequence
  Description of Artificial Sequence: Synthetic polypeptide
QVQLQQPGAELVKPGASVKLSCKSSGYHFTSYWMHWVKQRPGQGLEWIGVIHPNSGSINYNEKFESKATLTVDKSSSTAYMQLSSLTSEDSAVYYCAGERDSTEVLPMDYWGQGTSVTVSS

SEQ ID NO: 9 - protein, 10 aa, Artificial Sequence
  Description of Artificial Sequence: Synthetic peptide
GYHFTSYWMH

SEQ ID NO: 10 - protein, 17 aa, Artificial Sequence
  Description of Artificial Sequence: Synthetic peptide
VIHPNSGSINYNEKFES

SEQ ID NO: 11 - protein, 12 aa, Artificial Sequence
  Description of Artificial Sequence: Synthetic peptide
ERDSTEVLPMDY

SEQ ID NO: 12 - DNA, 321 bp, Artificial Sequence
  Description of Artificial Sequence: Synthetic polynucleotide
gatgtccagataacccagtctccatcttatcttgctgcatctcctggagaaaccattactattaattgcagggcaagtaagagcattaacaaatatttagcctggtatcaagagaaacctgggaaaactaataagcttcttatctactctggatccactttgcaatctggaattccatcaaggttcagtggcagtggatctggtacagatttcactctcaccatcagtagcctggagcctgaagattttgcaatgtattactgtcaacaacataatgaatacccgctcacgttcggtgctgggaccaagctggagctgaaa

SEQ ID NO: 13 - DNA, 363 bp, Artificial Sequence
  Description of Artificial Sequence: Synthetic polynucleotide
caggtccaactgcagcagcctggggctgagctggtaaagcctggggcttcagtgaagttgtcctgcaagtcttctggctaccatttcaccagctactggatgcactgggtgaagcagaggcctggacaaggccttgagtggattggagtgattcatcctaatagtggtagtattaactacaatgagaagttcgagagcaaggccacactgactgtagacaaatcctccagcacagcctacatgcaactcagcagcctgacatctgaggactcggcggtctattattgtgcaggagagagagattctacggaggttctccctatggactactggggtcaaggaacctcagtcaccgtctcctca

SEQ ID NO: 14-15 - skipped (2 entries)

SEQ ID NO: 16 - protein, 31 aa, Homo sapiens
GLFQVVSGGMVLQLQQGDQVWVEKDPKKGHI

SEQ ID NO: 17 - protein, 26 aa, Homo sapiens
GLFQVVSGGMVLQLQQGDQVWVEKDP

SEQ ID NO: 18 - protein, 20 aa, Homo sapiens
SGGMVLQLQQGDQVWVEKDP

SEQ ID NO: 19 - protein, 18 aa, Homo sapiens
SGGMVLQLQQGDQVWVEK

SEQ ID NO: 20 - protein, 23 aa, Homo sapiens
WLAVNDYYDMVGIQGSDSVFSGF

SEQ ID NO: 21 - protein, 16 aa, Homo sapiens
YDMVGIQGSDSVFSGF

SEQ ID NO: 22 - protein, 8 aa, Homo sapiens
YDMVGIQG

SEQ ID NO: 23 - protein, 23 aa, Homo sapiens
HTANLCVLLYRSGVKVVTFCGHT

SEQ ID NO: 24 - protein, 9 aa, Homo sapiens
RSGVKVVTF

SEQ ID NO: 25-30 - skipped (6 entries)

SEQ ID NO: 31 - protein, 121 aa, Artificial Sequence [sequence omitted]

SEQ ID NO: 32 - protein, 121 aa, Artificial Sequence [sequence omitted]

SEQ ID NO: 33 - protein, 121 aa, Artificial Sequence
  Description of Artificial Sequence: Synthetic polypeptide
QVQLVQSGAELKKPGASVKVSCKSSGYHFTSYWMHWVKQAPGQGLEWIGVIHPNSGSINYNEKFESRVTITVDKSTSTAYMELSSLRSEDTAVYYCAGERDSTEVLPMDYWGQGTTVTVSS

SEQ ID NO: 34 - protein, 121 aa, Artificial Sequence [sequence omitted]

SEQ ID NO: 35 - protein, 107 aa, Artificial Sequence [sequence omitted]

SEQ ID NO: 36 - protein, 107 aa, Artificial Sequence [sequence omitted]

SEQ ID NO: 37 - protein, 107 aa, Artificial Sequence
  Description of Artificial Sequence: Synthetic polypeptide
DVQITQSPSSLSASLGERATINCRASKSINKYLAWYQQKPGKAPKLLIYSGSTLQSGIPARFSGSGSGTDFTLTISSLEPEDFAMYYCQQHNEYPLTFGQGTKLEIK

SEQ ID NO: 38 - protein, 107 aa, Artificial Sequence [sequence omitted]

SEQ ID NO: 39-46 - skipped (8 entries)

SEQ ID NO: 47 - protein, 327 aa, Homo sapiens
ASTKGPSVFPLAPCSRSTSESTAALGCLVKDYFPEPVTVSWNSGALTSGVHTFPAVLQSSGLYSLSSVVTVPSSSLGTKTYTCNVDHKPSNTKVDKRVESKYGPPCPPCPAPEFEGGPSVFLFPPKPKDTLMISRTPEVTCVVVDVSQEDPEVQFNWYVDGVEVHNAKTKPREEQFNSTYRVVSVLTVLHQDWLNGKEYKCKVSNKGLPSSIEKTISKAKGQPREPQVYTLPPSQEEMTKNQVSLTCLVKGFYPSDIAVEWESNGQPENNYKTTPPVLDSDGSFFLYSRLTVDKSRWQEGNVFSCSVMHEALHNHYTQKSLSLSLGK

SEQ ID NO: 48-50 - skipped (3 entries)

SEQ ID NO: 51 - protein, 12 aa, Artificial Sequence
  Description of Artificial Sequence: Synthetic peptide
SSVSSSYLHWYQ

SEQ ID NO: 52 - protein, 10 aa, Artificial Sequence
  Description of Artificial Sequence: Synthetic peptide
STSNLASGVP

SEQ ID NO: 53 - protein, 10 aa, Artificial Sequence
  Description of Artificial Sequence: Synthetic peptide
HQYYRLPPIT

SEQ ID NO: 54 - protein, 12 aa, Artificial Sequence
  Description of Artificial Sequence: Synthetic peptide
GFTFSNYAMSWV

SEQ ID NO: 55 - protein, 10 aa, Artificial Sequence
  Description of Artificial Sequence: Synthetic peptide
ISSGGSHTYY

SEQ ID NO: 56 - protein, 11 aa, Artificial Sequence
  Description of Artificial Sequence: Synthetic peptide
ARLFTGYAMDY

SEQ ID NO: 57 - protein, 109 aa, Artificial Sequence
  Description of Artificial Sequence: Synthetic polypeptide
DIVMTQTTAIMSASLGERVTMTCTASSSVSSSYLHWYQQKPGSSPKLWIYSTSNLASGVPARFSGSGSGTFYSLTISSMEAEDDATYYCHQYYRLPPITFGAGTKLELK

SEQ ID NO: 58 - protein, 115 aa, Artificial Sequence
  Description of Artificial Sequence: Synthetic polypeptide
QVKLEESGGALVKPGGSLKLSCAASGFTFSNYAMSWVRQIPEKRLEWVATISSGGSHTYYLDSVKGRFTISRDNARDTLYLQMSSLRSEDTALYYCARLFTGYAMDYWGQGTSVT

SEQ ID NO: 59-61 - skipped (3 entries)

SEQ ID NO: 62 - protein, 12 aa, Artificial Sequence
  Description of Artificial Sequence: Synthetic peptide
TASSSVSSSYLH

SEQ ID NO: 63 - protein, 7 aa, Artificial Sequence
  Description of Artificial Sequence: Synthetic peptide
STSNLAS

SEQ ID NO: 64 - protein, 5 aa, Artificial Sequence
  Description of Artificial Sequence: Synthetic peptide
NYAMS

SEQ ID NO: 65 - protein, 17 aa, Artificial Sequence
  Description of Artificial Sequence: Synthetic peptide
TISSGGSHTYYLDSVKG

SEQ ID NO: 66 - protein, 9 aa, Artificial Sequence
  Description of Artificial Sequence: Synthetic peptide
LFTGYAMDY

SEQ ID NO: 67 - protein, 109 aa, Artificial Sequence
  Description of Artificial Sequence: Synthetic polypeptide
QIVLTQSPAIMSASLGERVTMTCTASSSVSSSYLHWYQQKPGSSPKLWIYSTSNLASGVPARFSGSGSGTFYSLTISSMEAEDDATYYCHQYYRLPPITFGAGTKLELK

SEQ ID NO: 68 - protein, 118 aa, Artificial Sequence
  Description of Artificial Sequence: Synthetic polypeptide
EVMLVESGGALVKPGGSLKLSCAASGFTFSNYAMSWVRQIPEKRLEWVATISSGGSHTYYLDSVKGRFTISRDNARDTLYLQMSSLRSEDTALYYCARLFTGYAMDYWGQGTSVTVSS

SEQ ID NO: 69 - DNA, 20 bp, Artificial Sequence
  Description of Artificial Sequence: Synthetic primer
ctgagactggaggcaaccat

SEQ ID NO: 70 - DNA, 20 bp, Artificial Sequence
  Description of Artificial Sequence: Synthetic primer
gatatctccttcgcgcagac

SEQ ID NO: 71 - DNA, 20 bp, Artificial Sequence
  Description of Artificial Sequence: Synthetic primer
aaatggtgaaggtcggtgtg

SEQ ID NO: 72 - DNA, 18 bp, Artificial Sequence
  Description of Artificial Sequence: Synthetic primer
tgaaggggtcgttgatgg